European Patent Application EP 4 183 407 A1, published May 24, 2023. Title: Therapeutic use of a glucagon derivative or a conjugate thereof for liver disease. Applicant: HANMI PHARM. CO., LTD. The sequence listing filed with the application follows.

SEQUENCE LISTING (70 sequences)

SEQ ID NO: 1 - protein, 29 aa, homo sapiens
HSQGTFTSDYSKYLDSRRAQDFVQWLMNT

SEQ ID NO: 2 - protein, 29 aa, Artificial Sequence
  glucagon derivative
HSQGTFTSDYSKYLDCDRAQDFVQWLMNT

SEQ ID NO: 3 - protein, 29 aa, Artificial Sequence
  glucagon derivative
HSQGTFTSDYSKYLDCERAQDFVQWLMNT

SEQ ID NO: 4 - protein, 29 aa, Artificial Sequence
  glucagon derivative
HSQGTFTSDYSKYLDSCDAQDFVQWLMNT

SEQ ID NO: 5 - protein, 29 aa, Artificial Sequence
  glucagon derivative
HSQGTFTSDYSKYLDSCEAQDFVQWLMNT

SEQ ID NO: 6 - protein, 29 aa, Artificial Sequence
  glucagon derivative
HSQGTFTSDYSKYLDSCEADDFVQWLMNT

SEQ ID NO: 7 - protein, 29 aa, Artificial Sequence
  glucagon derivative
YSQGTFTSDYSKYLDSCEADDFVQWLMNT

SEQ ID NO: 8 - protein, 29 aa, Artificial Sequence
  glucagon derivative
  MISC_FEATURE (2): Xaa is aminoisobutyric acid (Aib)
YXQGTFTSDYSKYLDSCDAQDFVQWLINT

SEQ ID NO: 9 - protein, 29 aa, Artificial Sequence
  glucagon derivative
  MISC_FEATURE (2): Xaa is aminoisobutyric acid (Aib)
YXQGTFTSDYSKYLDSCDAQDFVVWLINT

SEQ ID NO: 10 - protein, 29 aa, Artificial Sequence
  glucagon derivative
  MISC_FEATURE (2): Xaa is aminoisobutyric acid (Aib)
YXQGTFTSDYSKYLDSCDADDFVVWLINT

SEQ ID NO: 11 - protein, 29 aa, Artificial Sequence
  glucagon derivative
  MISC_FEATURE (2): Xaa is aminoisobutyric acid (Aib)
YXQGTFTSDYSKYLDEKCAKEFVQWLMNT

SEQ ID NO: 12 - protein, 30 aa, Artificial Sequence
  glucagon derivative
  MISC_FEATURE (2): Xaa is aminoisobutyric acid (Aib)
  MISC_FEATURE (16)..(20): amino acids at positions 16 and 20 form a ring
YXQGTFTSDYSKYLDEKRAKEFVQWLMNTC

SEQ ID NO: 13 - protein, 29 aa, Artificial Sequence
  glucagon derivative
  MISC_FEATURE (2): Xaa is aminoisobutyric acid (Aib)
YXQGTFTSDYSCYLDSRRAQDFVQWLMNT

SEQ ID NO: 14 - protein, 29 aa, Artificial Sequence
  glucagon derivative
  MISC_FEATURE (2): Xaa is aminoisobutyric acid (Aib)
YXQGTFTSDYSKYLDCKRAKEFVQWLMNT

SEQ ID NO: 15 - protein, 29 aa, Artificial Sequence
  glucagon derivative
  MISC_FEATURE (2): Xaa is aminoisobutyric acid (Aib)
YXQGTFTSDYSKYLCEKRAQDFVVWLMNT

SEQ ID NO: 16 - protein, 29 aa, Artificial Sequence
  glucagon derivative
  MISC_FEATURE (2): Xaa is aminoisobutyric acid (Aib)
YXQGTFTSDYSKYLDCRRAQVFVQWLMRT

SEQ ID NO: 17 - protein, 29 aa, Artificial Sequence
  glucagon derivative
  MISC_FEATURE (2): Xaa is aminoisobutyric acid (Aib)
YXQGTFTSDYSKYLDCVRAQDFVQWLMRT

SEQ ID NO: 18 - protein, 29 aa, Artificial Sequence
  glucagon derivative
  MISC_FEATURE (2): Xaa is aminoisobutyric acid (Aib)
YXQGTFTSDYSKYLDSRRACDFRLWLMNT

SEQ ID NO: 19 - protein, 29 aa, Artificial Sequence
  glucagon derivative
  MISC_FEATURE (2): Xaa is aminoisobutyric acid (Aib)
  MISC_FEATURE (16)..(20): amino acids at positions 16 and 20 form a ring
YXQGTFTSDYSKYLCEKRAKEFVQWLMNT

SEQ ID NO: 20 - protein, 29 aa, Artificial Sequence
  glucagon derivative
  MISC_FEATURE (2): Xaa is aminoisobutyric acid (Aib)
  MISC_FEATURE (16)..(20): amino acids at positions 16 and 20 form a ring
YXQGTFTSDYSKYLDECRAKEFVQWLMNT

SEQ ID NO: 21 - protein, 29 aa, Artificial Sequence
  glucagon derivative
  MISC_FEATURE (2): Xaa is aminoisobutyric acid (Aib)
  MISC_FEATURE (16)..(20): amino acids at positions 16 and 20 form a ring
YXQGTFTSDYSKYLDEKCAKEFVQWLMNT

SEQ ID NO: 22 - protein, 29 aa, Artificial Sequence
  glucagon derivative
  MISC_FEATURE (2): Xaa is aminoisobutyric acid (Aib)
  MISC_FEATURE (16)..(20): amino acids at positions 16 and 20 form a ring
YXQGTFTSDYSKYLDEKRCKEFVQWLMNT

SEQ ID NO: 23 - protein, 29 aa, Artificial Sequence
  glucagon derivative
  MISC_FEATURE (2): Xaa is aminoisobutyric acid (Aib)
  MISC_FEATURE (16)..(20): amino acids at positions 16 and 20 form a ring
YXQGTFTSDYSKYCDEKRAKEFVQWLMNT

SEQ ID NO: 24 - protein, 29 aa, Artificial Sequence
  glucagon derivative
  MISC_FEATURE (2): Xaa is aminoisobutyric acid (Aib)
  MISC_FEATURE (16)..(20): amino acids at positions 16 and 20 form a ring
YXQGTFTSDYSKCLDEKRAKEFVQWLMNT

SEQ ID NO: 25 - protein, 29 aa, Artificial Sequence
  glucagon derivative
  MISC_FEATURE (2): Xaa is aminoisobutyric acid (Aib)
  MISC_FEATURE (16)..(20): amino acids at positions 16 and 20 form a ring
YXQGTFTSDYSKYLDEKRAKCFVQWLMNT

SEQ ID NO: 26 - protein, 29 aa, Artificial Sequence
  glucagon derivative
  MISC_FEATURE (2): Xaa is aminoisobutyric acid (Aib)
  MISC_FEATURE (16)..(20): amino acids at positions 16 and 20 form a ring
WXQGTFTSDYSKYLDECRAKDFVQWLMNT

SEQ ID NO: 27 - protein, 29 aa, Artificial Sequence
  glucagon derivative
  MISC_FEATURE (2): Xaa is aminoisobutyric acid (Aib)
  MISC_FEATURE (16)..(20): amino acids at positions 16 and 20 form a ring
YXQGTFVSDYSKYLDECRAKDFVQWLMNT

SEQ ID NO: 28 - protein, 29 aa, Artificial Sequence
  glucagon derivative
  MISC_FEATURE (2): Xaa is aminoisobutyric acid (Aib)
  MISC_FEATURE (16)..(20): amino acids at positions 16 and 20 form a ring
WXQGTFVSDYSKYLDECRAKDFVQWLMNT

SEQ ID NO: 29 - protein, 29 aa, Artificial Sequence
  glucagon derivative
  MISC_FEATURE (2): Xaa is aminoisobutyric acid (Aib)
  MISC_FEATURE (16)..(20): amino acids at positions 16 and 20 form a ring
YXQGTFTSDYSKCLDERRAKDFVQWLMNT

SEQ ID NO: 30 - protein, 29 aa, Artificial Sequence
  glucagon derivative
  MISC_FEATURE (2): Xaa is aminoisobutyric acid (Aib)
  MISC_FEATURE (16)..(20): amino acids at positions 16 and 20 form a ring
WXQGTFTSDYSKCLDERRAKDFVQWLMNT

SEQ ID NO: 31 - protein, 29 aa, Artificial Sequence
  glucagon derivative
  MISC_FEATURE (2): Xaa is aminoisobutyric acid (Aib)
  MISC_FEATURE (17)..(21): amino acids at positions 17 and 21 form a ring
YXQGTFTSDYSKYLDCKRAKEFVQWLMNT

SEQ ID NO: 32 - protein, 28 aa, Artificial Sequence
  glucagon derivative
  MISC_FEATURE (15)..(19): amino acids at positions 15 and 19 form a ring
SQGTFTSDYSKYLDECRAKEFVQWLMNT

SEQ ID NO: 33 - protein, 29 aa, Artificial Sequence
  glucagon derivative
  MISC_FEATURE (2): Xaa is aminoisobutyric acid (Aib)
YXQGTFTSDYSKYLDSRRAQDFVQWLMNT

SEQ ID NO: 34 - protein, 29 aa, Artificial Sequence
  glucagon derivative
  MISC_FEATURE (2): Xaa is aminoisobutyric acid (Aib)
  MISC_FEATURE (16)..(20): amino acids at positions 16 and 20 form a ring
WXQGTFTSDYSKYCDERRAKEFVQWLMNT

SEQ ID NO: 35 - protein, 29 aa, Artificial Sequence
  glucagon derivative
  MISC_FEATURE (2): Xaa is aminoisobutyric acid (Aib)
  MISC_FEATURE (16)..(20): amino acids at positions 16 and 20 form a ring
YXQGTFTSDYSKYCDERRAKEFVQWLMNT

SEQ ID NO: 36 - protein, 29 aa, Artificial Sequence
  glucagon derivative
  MISC_FEATURE (2): Xaa is aminoisobutyric acid (Aib)
  MISC_FEATURE (16)..(20): amino acids at positions 16 and 20 form a ring
YXQGTFTSDCSKYLDERRAKEFVQWLMNT

SEQ ID NO: 37 - protein, 30 aa, Artificial Sequence
  glucagon derivative
  MISC_FEATURE (2): Xaa is aminoisobutyric acid (Aib)
  MISC_FEATURE (16)..(20): amino acids at positions 16 and 20 form a ring
YXQGTFTSDYSKYLDERRAKEFVQWLMNTC

SEQ ID NO: 38 - protein, 29 aa, Artificial Sequence
  glucagon derivative
  MISC_FEATURE (2): Xaa is aminoisobutyric acid (Aib)
  MISC_FEATURE (16)..(20): amino acids at positions 16 and 20 form a ring
YXQGTFCSDYSKYLDERRAKEFVQWLMNT

SEQ ID NO: 39 - protein, 29 aa, Artificial Sequence
  glucagon derivative
  MISC_FEATURE (2): Xaa is aminoisobutyric acid (Aib)
  MISC_FEATURE (16)..(20): amino acids at positions 16 and 20 form a ring
YXQGTFVSDCSKYLDERRAKDFVQWLMNT

SEQ ID NO: 40 - protein, 30 aa, Artificial Sequence
  glucagon derivative
  MISC_FEATURE (2): Xaa is aminoisobutyric acid (Aib)
  MISC_FEATURE (16)..(20): amino acids at positions 16 and 20 form a ring
YXQGTFVSDYSKYLDERRAKDFVQWLMNTC

SEQ ID NO: 41 - protein, 29 aa, Artificial Sequence
  glucagon derivative
  MISC_FEATURE (2): Xaa is aminoisobutyric acid (Aib)
  MISC_FEATURE (16)..(20): amino acids at positions 16 and 20 form a ring
YXQGTFCSDYSKYLDERRAKDFVQWLMNT

SEQ ID NO: 42 - protein, 29 aa, Artificial Sequence
  glucagon derivative
  MISC_FEATURE (2): Xaa is aminoisobutyric acid (Aib)
YXQGTFCSDYSKYLDSRRAQDFVQWLMNT

SEQ ID NO: 43 - protein, 29 aa, Artificial Sequence
  glucagon derivative
  MISC_FEATURE (2): Xaa is aminoisobutyric acid (Aib)
YXQGTFTSDCSKYLDSRRAQDFVQWLMNT

SEQ ID NO: 44 - protein, 30 aa, Artificial Sequence
  glucagon derivative
  MISC_FEATURE (2): Xaa is aminoisobutyric acid (Aib)
YXQGTFTSDYSKYLDSRRAQDFVQWLMNTC

SEQ ID NO: 45 - protein, 29 aa, Artificial Sequence
  glucagon derivative
  MISC_FEATURE (2): Xaa is aminoisobutyric acid (Aib)
YXQGTFTSDYSCYLDEKRAKEFVQWLMNT

SEQ ID NO: 46 - protein, 30 aa, Artificial Sequence
  General Formula 1
  MISC_FEATURE (2): Xaa is aminoisobutyric acid (Aib)
  MISC_FEATURE (7): Xaa is threonine, valine, or cysteine
  MISC_FEATURE (14): Xaa is leucine or cysteine
  MISC_FEATURE (16): Xaa is glutamic acid, or serine
  MISC_FEATURE (17): Xaa is lysine, arginine, or cysteine
  MISC_FEATURE (19): Xaa is alanine, or cysteine
  MISC_FEATURE (20): Xaa is lysine, or glutamine
  MISC_FEATURE (21): Xaa is aspartic acid, or glutamic acid
  MISC_FEATURE (30): Xaa is cysteine, or is absent
YXQGTFXSDYSKYXDXXRXXXFVQWLMNTX

SEQ ID NO: 47 - DNA, 34 bp, Artificial Sequence
  Primer
cagcgacaccgaccgtccccccgtacttaaggcc

SEQ ID NO: 48 - DNA, 32 bp, Artificial Sequence
  Primer
ctaaccgactctcggggaagactgagctcgcc

SEQ ID NO: 49 - protein, 12 aa, homo sapiens
ESKYGPPCPSCP

SEQ ID NO: 50 - protein, 11 aa, Artificial Sequence
  Variant of hinge region
ESKYGPPPSCP

SEQ ID NO: 51 - protein, 11 aa, Artificial Sequence
  Variant of hinge region
ESKYGPPCPSP

SEQ ID NO: 52 - protein, 10 aa, Artificial Sequence
  Variant of hinge region
ESKYGPPCPS

SEQ ID NO: 53 - protein, 10 aa, Artificial Sequence
  Variant of hinge region
ESKYGPPCPP

SEQ ID NO: 54 - protein, 8 aa, Artificial Sequence
  Variant of hinge region
KYGPPCPS

SEQ ID NO: 55 - protein, 8 aa, Artificial Sequence
  Variant of hinge region
ESKYGPPC

SEQ ID NO: 56 - protein, 7 aa, Artificial Sequence
  Variant of hinge region
EKYGPPC

SEQ ID NO: 57 - protein, 6 aa, Artificial Sequence
  Variant of hinge region
ESPSCP

SEQ ID NO: 58 - protein, 5 aa, Artificial Sequence
  Variant of hinge region
EPSCP

SEQ ID NO: 59 - protein, 4 aa, Artificial Sequence
  Variant of hinge region
PSCP

SEQ ID NO: 60 - protein, 10 aa, Artificial Sequence
  Variant of hinge region
ESKYGPPSCP

SEQ ID NO: 61 - protein, 9 aa, Artificial Sequence
  Variant of hinge region
KYGPPPSCP

SEQ ID NO: 62 - protein, 9 aa, Artificial Sequence
  Variant of hinge region
ESKYGPSCP

SEQ ID NO: 63 - protein, 8 aa, Artificial Sequence
  Variant of hinge region
ESKYGPPC

SEQ ID NO: 64 - protein, 7 aa, Artificial Sequence
  Variant of hinge region
KYGPPCP

SEQ ID NO: 65 - protein, 7 aa, Artificial Sequence
  Variant of hinge region
ESKPSCP

SEQ ID NO: 66 - protein, 6 aa, Artificial Sequence
  Variant of hinge region
ESPSCP

SEQ ID NO: 67 - protein, 4 aa, Artificial Sequence
  Variant of hinge region
EPSC

SEQ ID NO: 68 - protein, 3 aa, Artificial Sequence
  Variant of hinge region
SCP

SEQ ID NO: 69 - protein, 221 aa, homo sapiens
PSCPAPEFLGGPSVFLFPPKPKDTLMISRTPEVTCVVVDVSQEDPEVQFNWYVDGVEVHNAKTKPREEQFNSTYRVVSVLTVLHQDWLNGKEYKCKVSNKGLPSSIEKTISKAKGQPREPQVYTLPPSQEEMTKNQVSLTCLVKGFYPSDIAVEWESNGQPENNYKTTPPVLDSDGSFFLYSRLTVDKSRWQEGNVFSCSVMHEALHNHYTQKSLSLSLGK

SEQ ID NO: 70 - protein, 442 aa, Homo sapiens
  MISC_FEATURE (1)..(442): Amino acids at position 1 to 442 form Human Immunoglobulin G4 Fc Fragment (homodimer)
  MISC_FEATURE (1)..(221): Amino acids at position 1 to 221 form one monomer
  MISC_FEATURE (222)..(442): Amino acids at position 222 to 442 form one monomer
  DISULFID (3)..(224): Amino acids at position 3 and position 224 form an inter-disulfide bond
  DISULFID (35)..(95): Amino acids at position 35 and position 95 form an intra-chain disulfide bond
  DISULFID (141)..(199): Amino acids at position 141 and position 199 form an intra-chain disulfide bond
  DISULFID (256)..(316): Amino acids at position 256 and position 316 form an intra-chain disulfide bond
  DISULFID (362)..(420): Amino acids at position 362 and position 420 form an intra-chain disulfide bond
PSCPAPEFLGGPSVFLFPPKPKDTLMISRTPEVTCVVVDVSQEDPEVQFNWYVDGVEVHNAKTKPREEQFNSTYRVVSVLTVLHQDWLNGKEYKCKVSNKGLPSSIEKTISKAKGQPREPQVYTLPPSQEEMTKNQVSLTCLVKGFYPSDIAVEWESNGQPENNYKTTPPVLDSDGSFFLYSRLTVDKSRWQEGNVFSCSVMHEALHNHYTQKSLSLSLGKPSCPAPEFLGGPSVFLFPPKPKDTLMISRTPEVTCVVVDVSQEDPEVQFNWYVDGVEVHNAKTKPREEQFNSTYRVVSVLTVLHQDWLNGKEYKCKVSNKGLPSSIEKTISKAKGQPREPQVYTLPPSQEEMTKNQVSLTCLVKGFYPSDIAVEWESNGQPENNYKTTPPVLDSDGSFFLYSRLTVDKSRWQEGNVFSCSVMHEALHNHYTQKSLSLSLGK